European Patent Specification EP 3 606 615 B1, published January 7, 2026. Title: HAIR CARE COMPOSITIONS. Applicant: Yissum Research Development Company of the Hebrew University of Jerusalem Ltd. Smart Resilin Ltd. SHOSEYOV, Oded SHALEV, Roni BARUCH-SHARON, Sigal BEN SHALOM, Tal NUTTMAN-NESIAL, Liron. The sequence listing filed with the application follows.

SEQUENCE LISTING (21 sequences)

SEQ ID NO: 1 - protein, 324 aa, Artificial sequence
  Drosophila melanogaster derived resilin exon 1
MGPEPPVNSYLPPSDSYGAPGQSGPGGRPSDSYGAPGGGNGGRPSDSYGAPGQGQGQGQGQGGYAGKPSDTYGAPGGGNGNGGRPSSSYGAPGGGNGGRPSDTYGAPGGGNGGRPSDTYGAPGGGGNGNGGRPSSSYGAPGQGQGNGNGGRSSSSYGAPGGGNGGRPSDTYGAPGGGNGGRPSDTYGAPGGGNNGGRPSSSYGAPGGGNGGRPSDTYGAPGGGNGNGSGGRPSSSYGAPGQGQGGFGGRPSDSYGAPGQNQKPSDSYGAPGSGNGNGGRPSSSYGAPGSGPGGRPSDSYGPPASGSGAGGAGGSGPGGADYDND

SEQ ID NO: 2 - protein, 323 aa, Artificial sequence
  Drosophila melanogaster derived resilin exon 1
GPEPPVNSYLPPSDSYGAPGQSGPGGRPSDSYGAPGGGNGGRPSDSYGAPGQGQGQGQGQGGYAGKPSDTYGAPGGGNGNGGRPSSSYGAPGGGNGGRPSDTYGAPGGGNGGRPSDTYGAPGGGGNGNGGRPSSSYGAPGQGQGNGNGGRSSSSYGAPGGGNGGRPSDTYGAPGGGNGGRPSDTYGAPGGGNNGGRPSSSYGAPGGGNGGRPSDTYGAPGGGNGNGSGGRPSSSYGAPGQGQGGFGGRPSDSYGAPGQNQKPSDSYGAPGSGNGNGGRPSSSYGAPGSGPGGRPSDSYGPPASGSGAGGAGGSGPGGADYDND

SEQ ID NO: 3 - protein, 62 aa, Artificial sequence
  Chitin binding sequence
EPAKYEFNYQVEDAPSGLSFGHSEMRDGDFTTGQYNVLLPDGRKQIVEYEADQQGYRPQIRY

SEQ ID NO: 4 - protein, 15 aa, Artificial sequence
  Resilin repeating unit
GGRPSDSYGAPGGGN

SEQ ID NO: 5 - protein, 9 aa, Artificial sequence
  Resilin repeating unit
GRPSDSYGA

SEQ ID NO: 6 - protein, 74 aa, Artificial sequence
  Chitin binding sequence
PAKYEFNYQVEDAPSGLSFGHSEMRDGDFTTGQYNVLLPDGRKQIVEYEADQQGYRPQIRYEGDANDGSGPSGP

SEQ ID NO: 7 - DNA, 900 bp, Artificial sequence
  Examples of polynucleotides which can be used to express resilin
agctatggagcaccgggtcagagtggtcccggcggcaggccgtcggattcctatggagctcctggtggtggaaacggtggacggccctcagacagctatggcgctccaggccagggtcaaggacagggacaaggacaaggtggatatgcaggcaagccctcagatacctatggagctcctggtggtggaaatggcaacggaggtcgtccatcgagcagctatggcgctcctggcggtggaaacggtggtcgtccttcggatacctacggtgctcctggtggcggaaatggtggacgcccatcggacacttatggtgctcctggtggtggtggaaatggcaacggcggacgaccttcaagcagctatggagctcctggtcaaggacaaggcaacggaaatggcggtcgctcatcgagcagctatggtgctcctggcggtggaaacggcggtcgtccttcggatacctacggtgctcccggtggtggaaacggtggtcgtccttcggatacttacggcgctcctggtggcggcaataatggcggtcgtccctcaagcagctacggcgctcctggtggtggaaacggtggtcgtccatctgacacctatggcgctcctggtggcggtaacggaaacggcagcggtggtcgtccttcaagcagctatggagctcctggtcagggccaaggtggatttggtggtcgtccatcggactcctatggtgctcctggtcagaaccaaaaaccatcagattcatatggcgcccctggtagcggcaatggcaacggcggacgtccttcgagcagctatggagctccaggctcaggacctggtggccgaccctccgactcctacggacccccagcttctggatcgggagcaggtggcgctggaggcagtgga

SEQ ID NO: 8 - DNA, 1080 bp, Artificial sequence
  An exemplary DNA sequence of 6H-tagged resilin (exon 1)
atgtcgtactaccatcaccatcaccatcacgattacgatatcccaacgaccgaaaacctgtattttcagggcgccatgggaccggagccaccagttaactcgtatctacctccgtccgatagctatggagcaccgggtcagagtggtcccggcggcaggccgtcggattcctatggagctcctggtggtggaaacggtggacggccctcagacagctatggcgctccaggccagggtcaaggacagggacaaggacaaggtggatatgcaggcaagccctcagatacctatggagctcctggtggtggaaatggcaacggaggtcgtccatcgagcagctatggcgctcctggcggtggaaacggtggtcgtccttcggatacctacggtgctcctggtggcggaaatggtggacgcccatcggacacttatggtgctcctggtggtggtggaaatggcaacggcggacgaccttcaagcagctatggagctcctggtcaaggacaaggcaacggaaatggcggtcgctcatcgagcagctatggtgctcctggcggtggaaacggcggtcgtccttcggatacctacggtgctcccggtggtggaaacggtggtcgtccttcggatacttacggcgctcctggtggcggcaataatggcggtcgtccctcaagcagctacggcgctcctggtggtggaaacggtggtcgtccatctgacacctatggcgctcctggtggcggtaacggaaacggcagcggtggtcgtccttcaagcagctatggagctcctggtcagggccaaggtggatttggtggtcgtccatcggactcctatggtgctcctggtcagaaccaaaaaccatcagattcatatggcgcccctggtagcggcaatggcaacggcggacgtccttcgagcagctatggagctccaggctcaggacctggtggccgaccctccgactcctacggacccccagcttctggatcgggagcaggtggcgctggaggcagtggacccggcggcgctgactacgataacgatgagggatccaatcactagtgaattcgcggccgc

SEQ ID NO: 9 - protein, 354 aa, Artificial sequence
  An exemplary [protein sequence of 6H-tagged resilin (exon 1)
MSYYHHHHHHDYDIPTTENLYFQGAMGPEPPVNSYLPPSDSYGAPGQSGPGGRPSDSYGAPGGGNGGRPSDSYGAPGQGQGQGQGQGGYAGKPSDTYGAPGGGNGNGGRPSSSYGAPGGGNGGRPSDTYGAPGGGNGGRPSDTYGAPGGGGNGNGGRPSSSYGAPGQGQGNGNGGRSSSSYGAPGGGNGGRPSDTYGAPGGGNGGRPSDTYGAPGGGNNGGRPSSSYGAPGGGNGGRPSDTYGAPGGGNGNGSGGRPSSSYGAPGQGQGGFGGRPSDSYGAPGQNQKPSDSYGAPGSGNGNGGRPSSSYGAPGSGPGGRPSDSYGPPASGSGAGGAGGSGPGGADYDNDEGSNH

SEQ ID NO: 10 - DNA, 1311 bp, Artificial sequence
  An exemplary DNA sequence of 6H-tagged resilin (exons 1 and 2)
catatgtcgtactaccatcaccatcaccatcacgattacgatatcccaacgaccgaaaacctgtattttcagggcgccatgggaccggagccaccagttaactcgtatctacctccgtccgatagctatggagcaccgggtcagagtggtcccggcggcaggccgtcggattcctatggagctcctggtggtggaaacggtggacggccctcagacagctatggcgctccaggccagggtcaaggacagggacaaggacaaggtggatatgcaggcaagccctcagatacctatggagctcctggtggtggaaatggcaacggaggtcgtccatcgagcagctatggcgctcctggcggtggaaacggtggtcgtccttcggatacctacggtgctcctggtggcggaaatggtggacgcccatcggacacttatggtgctcctggtggtggtggaaatggcaacggcggacgaccttcaagcagctatggagctcctggtcaaggacaaggcaacggaaatggcggtcgctcatcgagcagctatggtgctcctggcggtggaaacggcggtcgtccttcggatacctacggtgctcccggtggtggaaacggtggtcgtccttcggatacttacggcgctcctggtggcggcaataatggcggtcgtccctcaagcagctacggcgctcctggtggtggaaacggtggtcgtccatctgacacctatggcgctcctggtggcggtaacggaaacggcagcggtggtcgtccttcaagcagctatggagctcctggtcagggccaaggtggatttggtggtcgtccatcggactcctatggtgctcctggtcagaaccaaaaaccatcagattcatatggcgcccctggtagcggcaatggcaacggcggacgtccttcgagcagctatggagctccaggctcaggacctggtggccgaccctccgactcctacggacccccagcttctggatcgggagcaggtggcgctggaggcagtggacccggcggcgctgactacgataacgatgagcccgccaagtacgaatttaattaccaggttgaggacgcgcccagcggactctcgttcgggcattcagagatgcgcgacggtgacttcaccaccggccagtacaatgtcctgttgcccgacggaaggaagcaaattgtggagtatgaagccgaccagcagggctaccggccacagatccgctacgaaggcgatgccaacgatggcagtggtcccagcggtccttaaggatccgagctccgtcgacaagcttgcggccgc

SEQ ID NO: 11 - protein, 424 aa, Artificial sequence
  An exemplary protein sequence of 6H-tagged resilin (exons 1 and 2)
MSYYHHHHHHDYDIPTTENLYFQGAMGPEPPVNSYLPPSDSYGAPGQSGPGGRPSDSYGAPGGGNGGRPSDSYGAPGQGQGQGQGQGGYAGKPSDTYGAPGGGNGNGGRPSSSYGAPGGGNGGRPSDTYGAPGGGNGGRPSDTYGAPGGGGNGNGGRPSSSYGAPGQGQGNGNGGRSSSSYGAPGGGNGGRPSDTYGAPGGGNGGRPSDTYGAPGGGNNGGRPSSSYGAPGGGNGGRPSDTYGAPGGGNGNGSGGRPSSSYGAPGQGQGGFGGRPSDSYGAPGQNQKPSDSYGAPGSGNGNGGRPSSSYGAPGSGPGGRPSDSYGPPASGSGAGGAGGSGPGGADYDNDEPAKYEFNYQVEDAPSGLSFGHSEMRDGDFTTGQYNVLLPDGRKQIVEYEADQQGYRPQIRYEGDANDGSGPSGP

SEQ ID NO: 12 - DNA, 1580 bp, Artificial sequence
  An exemplary DNA sequence of 6H-tagged resilin (exon 1) fused to a cellulose-binding domain (CBD)
catatgtcgtactaccatcaccatcaccatcacgattacgatatcccaacgaccgaaaacctgtattttcagggcgccatgggaccggagccaccagttaactcgtatctacctccgtccgatagctatggagcaccgggtcagagtggtcccggcggcaggccgtcggattcctatggagctcctggtggtggaaacggtggacggccctcagacagctatggcgctccaggccagggtcaaggacagggacaaggacaaggtggatatgcaggcaagccctcagatacctatggagctcctggtggtggaaatggcaacggaggtcgtccatcgagcagctatggcgctcctggcggtggaaacggtggtcgtccttcggatacctacggtgctcctggtggcggaaatggtggacgcccatcggacacttatggtgctcctggtggtggtggaaatggcaacggcggacgaccttcaagcagctatggagctcctggtcaaggacaaggcaacggaaatggcggtcgctcatcgagcagctatggtgctcctggcggtggaaacggcggtcgtccttcggatacctacggtgctcccggtggtggaaacggtggtcgtccttcggatacttacggcgctcctggtggcggcaataatggcggtcgtccctcaagcagctacggcgctcctggtggtggaaacggtggtcgtccatctgacacctatggcgctcctggtggcggtaacggaaacggcagcggtggtcgtccttcaagcagctatggagctcctggtcagggccaaggtggatttggtggtcgtccatcggactcctatggtgctcctggtcagaaccaaaaaccatcagattcatatggcgcccctggtagcggcaatggcaacggcggacgtccttcgagcagctatggagctccaggctcaggacctggtggccgaccctccgactcctacggacccccagcttctggatcgggagcaggtggcgctggaggcagtggacccggcggcgctgactacgataacgatgaggggatccccgaccccggcatggcagcgacatcatcaatgtcagttgaattttacaactctaacaaatcagcacaaacaaactcaattacaccaataatcaaaattactaacacatctgacagtgatttaaatttaaatgacgtaaaagttagatattattacacaagtgatggtacacaaggacaaactttctggtgtgaccatgctggtgcattattaggaaatagctatgttgataacactagcaaagtgacagcaaacttcgttaaagaaacagcaagcccaacatcaacctatgatacatatgttgaatttggatttgcaagcggacgagctactcttaaaaaaggacaatttataactattcaaggaagaataacaaaatcagactggtcaaactacactcaaacaaatgactattcatttgatgcaagtagttcaacaccagttgtaaatccaaaagttacaggatatataggtggagctaaagtacttggtacagcaccataggatcgatccagatgtac

SEQ ID NO: 13 - protein, 519 aa, Artificial sequence
  An exemplary protein sequence of 6H-tagged resilin (exon 1) fused to a cellulose-binding domain (CBD)
MSYYHHHHHHDYDIPTTENLYFQGAMGPEPPVNSYLPPSDSYGAPGQSGPGGRPSDSYGAPGGGNGGRPSDSYGAPGQGQGQGQGQGGYAGKPSDTYGAPGGGNGNGGRPSSSYGAPGGGNGGRPSDTYGAPGGGNGGRPSDTYGAPGGGGNGNGGRPSSSYGAPGQGQGNGNGGRSSSSYGAPGGGNGGRPSDTYGAPGGGNGGRPSDTYGAPGGGNNGGRPSSSYGAPGGGNGGRPSDTYGAPGGGNGNGSGGRPSSSYGAPGQGQGGFGGRPSDSYGAPGQNQKPSDSYGAPGSGNGNGGRPSSSYGAPGSGPGGRPSDSYGPPASGSGAGGAGGSGPGGADYDNDEGIPDPGMAATSSMSVEFYNSNKSAQTNSITPIIKITNTSDSDLNLNDVKVRYYYTSDGTQGQTFWCDHAGALLGNSYVDNTSKVTANFVKETASPTSTYDTYVEFGFASGRATLKKGQFITIQGRITKSDWSNYTQTNDYSFDASSSTPVVNPKVTGYIGGAKVLGTAP

SEQ ID NO: 14 - DNA, 1620 bp, Artificial sequence
  An exemplary DNA sequence of 6H-tagged resilin (exon 1) fused to a cellulose-binding domain (CBD)
catatgtcgtactaccatcaccatcaccatcacgattacgatatcccaacgaccgaaaacctgtattttcagggcgccatggcagcgacatcatcaatgtcagttgaattttacaactctaacaaagcagcacaaacaaactcaattacaccaataatcaaaattactaacacagctgacagtgatttaaatttaaatgacgtaaaagttagatattattacacaagtgatggtacacaaggacaaactttctggggtgatcatgctggtgcattattaggaaatagctatgttgataacactggcaaagtgacagcaaacttcgttaaagaaacagcaagcccaacatcaacctatgatacatatgttgaatttggatttgcaagcggagcagctactcttaaaaaaggacaatttataactattcaaggaagaataacaaaatcagactggtcaaactacgctcagacaaatgactattcatttgatgcaagtagttcaacaccagttgtaaatccaaaagttacaggatatataggtggagctaaagtacttggtacagcaccaggtccagatgtaccatcttcaataattaatcctacttctgcaacatttgatccggagccaccagttaactcgtatctacctccgtccgatagctatggagcaccgggtcagagtggtcccggcggcaggccgtcggattcctatggagctcctggtggtggaaacggtggacggccctcagacagctatggcgctccaggccagggtcaaggacagggacaaggacaaggtggatatgcaggcaagccctcagatacctatggagctcctggtggtggaaatggcaacggaggtcgtccatcgagcagctatggcgctcctggcggtggaaacggtggtcgtccttcggatacctacggtgctcctggtggcggaaatggtggacgcccatcggacacttatggtgctcctggtggtggtggaaatggcaacggcggacgaccttcaagcagctatggagctcctggtcaaggacaaggcaacggaaatggcggtcgctcatcgagcagctatggtgctcctggcggtggaaacggcggtcgtccttcggatacctacggtgctcccggtggtggaaacggtggtcgtccttcggatacttacggcgctcctggtggcggcaataatggcggtcgtccctcaagcagctacggcgctcctggtggtggaaacggtggtcgtccatctgacacctatggcgctcctggtggcggtaacggaaacggcagcggtggtcgtccttcaagcagctatggagctcctggtcagggccaaggtggatttggtggtcgtccatcggactcctatggtgctcctggtcagaaccaaaaaccatcagattcatatggcgcccctggtagcggcaatggcaacggcggacgtccttcgagcagctatggagctccaggctcaggacctggtggccgaccctccgactcctacggacccccagcttctggatcgggagcaggtggcgctggaggcagtggacccggcggcgctgactacgataacgatgagtaaggatccgagctccgtcgacaagcttgcggc

SEQ ID NO: 15 - protein, 528 aa, Artificial sequence
  An exemplary protein sequence of 6H-tagged resilin (exon 1) fused to a cellulose-binding domain (CBD)
MSYYHHHHHHDYDIPTTENLYFQGAMAATSSMSVEFYNSNKAAQTNSITPIIKITNTADSDLNLNDVKVRYYYTSDGTQGQTFWGDHAGALLGNSYVDNTGKVTANFVKETASPTSTYDTYVEFGFASGAATLKKGQFITIQGRITKSDWSNYAQTNDYSFDASSSTPVVNPKVTGYIGGAKVLGTAPGPDVPSSIINPTSATFDPEPPVNSYLPPSDSYGAPGQSGPGGRPSDSYGAPGGGNGGRPSDSYGAPGQGQGQGQGQGGYAGKPSDTYGAPGGGNGNGGRPSSSYGAPGGGNGGRPSDTYGAPGGGNGGRPSDTYGAPGGGGNGNGGRPSSSYGAPGQGQGNGNGGRSSSSYGAPGGGNGGRPSDTYGAPGGGNGGRPSDTYGAPGGGNNGGRPSSSYGAPGGGNGGRPSDTYGAPGGGNGNGSGGRPSSSYGAPGQGQGGFGGRPSDSYGAPGQNQKPSDSYGAPGSGNGNGGRPSSSYGAPGSGPGGRPSDSYGPPASGSGAGGAGGSGPGGADYDNDE

SEQ ID NO: 16 - protein, 324 aa, Artificial sequence
  Resilin exon 1
GPEPPVNSYLPPSDSYGAPGQSGPGGRPSDSYGAPGGGNGGRPSDSYGAPGQGQGQGQGQGGYAGKPSDTYGAPGGGNGNGGRPSSSYGAPGGGNGGRPSDTYGAPGGGNGGRPSDTYGAPGGGGNGNGGRPSSSYGAPGQGQGNGNGGRSSSSYGAPGGGNGGRPSDTYGAPGGGNGGRPSDTYGAPGGGNNGGRPSSSYGAPGGGNGGRPSDTYGAPGGGNGNGSGGRPSSSYGAPGQGQGGFGGRPSDSYGAPGQNQKPSDSYGAPGSGNGNGGRPSSSYGAPGSGPGGRPSDSYGPPASGSGAGGAGGSGPGGADYDNDE

SEQ ID NO: 17 - protein, 180 aa, Artificial sequence
  Cellulose binding domain protein sequence
MAATSSMSVEFYNSNKAAQTNSITPIIKITNTADSDLNLNDVKVRYYYTSDGTQGQTFWGDHAGALLGNSYVDNTGKVTANFVKETASPTSTYDTYVEFGFASGAATLKKGQFITIQGRITKSDWSNYAQTNDYSFDASSSTPVVNPKVTGYIGGAKVLGTAPGPDVPSSIINPTSATFD

SEQ ID NO: 18 - protein, 163 aa, Artificial sequence
  Cellulose binding domain protein sequence
MAATSSMSVEFYNSNKAAQTNSITPIIKITNTADSDLNLNDVKVRYYYTSDGTQGQTFWGDHAGALLGNSYVDNTGKVTANFVKETASPTSTYDTYVEFGFASGAATLKKGQFITIQGRITKSDWSNYAQTNDYSFDASSSTPVVNPKVTGYIGGAKVLGTAP

SEQ ID NO: 19 - protein, 605 aa, Drosophila melanogaster
MVRPEPPVNSYLPPSDSYGAPGQSGPGGRPSDSYGAPGGGNGGRPSDSYGAPGQGQGQGQGQGGYAGKPSDTYGAPGGGNGNGGRPSSSYGAPGGGNGGRPSDTYGAPGGGNGGRPSDTYGAPGGGGNGNGGRPSSSYGAPGQGQGNGNGGRSSSSYGAPGGGNGGRPSDTYGAPGGGNGGRPSDTYGAPGGGNNGGRPSSSYGAPGGGNGGRPSDTYGAPGGGNGNGSGGRPSSSYGAPGQGQGGFGGRPSDSYGAPGQNQKPSDSYGAPGSGNGNGGRPSSSYGAPGSGPGGRPSDSYGPPASGSGAGGAGGSGPGGADYDNDEPAKYEFNYQVEDAPSGLSFGHSEMRDGDFTTGQYNVLLPDGRKQIVEYEADQQGYRPQIRYEGDANDGSGPSGPGGPGGQNLGADGYSSGRPGNGNGNGNGGYSGGRPGGQDLGPSGYSGGRPGGQDLGAGGYSNGKPGGQDLGPGGYSGGRPGGQDLGRDGYSGGRPGGQDLGASGYSNGRPGGNGNGGSDGGRVIIGGRVIGGQDGGDQGYSGGRPGGQDLGRDGYSSGRPGGRPGGNGQDSQDGQGYSSGRPGQGGRNGFGPGGQNGDNDGSGYRY

SEQ ID NO: 20 - protein, 7 aa, Artificial Sequence
  Resilin consensus amino acid sequence repeats
  misc_feature (2)..(3): Xaa can be any naturally occurring amino acid
  misc_feature (6)..(6): Xaa can be any naturally occurring amino acid
SXXYGXP

SEQ ID NO: 21 - protein, 1848 aa, Clostridium cellulovorans
MQKKKSLNLLLALMMVFALVLPSIPALAATSSMSVEFYNSNKSAQTNSITPIIKITNTSDSDLNLNDVKVRYYYTSDGTQGQTFWCDHAGALLGNSYVDNTSKVTANFVKETASPTSTYDTYVEFGFASGRATLKKGQFITIQGRITKSDWSNYTQTNDYSFDASSSTPVVNPKVTGYIGGAKVLGTAPGPDVPSSIINPTSATFDKNVTKQADVKTTMTLNGNTFKTITDANGTALNASTDYSVSGNDVTISKAYLAKQSVGTTTLNFNFSAGNPQKLVITVVDTPVEAVTATIGKVQVNAGETVAVPVNLTKVPAAGLATIELPLTFDSASLEVVSITAGDIVLNPSVNFSSTVSGSTIKLLFLDDTLGSQLITKDGVFATITFKAKAITGTTAKVTSVKLAGTPVVGDAQLQEKPCAVNPGTVTINPIDNRMQISVGTATVKAGEIAAVPVTLTSVPSTGIATAEAQVSFDATLLEVASVTAGDIVLNPTVNFSYTVNGNVIKLLFLDDTLGSQLISKDGVFVTINFKAKAVTSTVTTPVTVSGTPVFADGTLAEVQSKTAAGSVTINIGDPILEPTISPVTATFDKKAPADVATTMTLNGYTFNGITGLTTSDYSISGNVVKISQAYLAKQPVGDLTLTFNFSNGNKTATAKLVVSIKDAPKTVTATVGTATVNAGETVAVPVTLSNVSGISTAELQLSFDATLLEVVSITAGDIVLNPSVNFSSVVNGSTIKLLFLDDTLGSQLISKDGVFATINFKAKSVTSTVTTPVKVSGTPVFADGTLAELSYETVAGSVTINAIGPVKTVTATVGTATVKSGETVAVPVTLSNVPGIATAELQLSFDATLLEVASITVGDIVLNPSVNFSSVVNGSTIKLLFLDDTLGSQLISKDGVLATINFKAKTVTSTVTTPVAVSGTPVFADGTLAELQSKTVAGSVTIEPSQPVKTVTATVGTATVKSGETVAVPVTLSNVPGIATAELQVGFDATLLEVASITVGDIVLNPSVNFSSVVNGSTIKLLFLDDTLGSQLISKDGVLATINFKAKTVTSKVTTPVAVSGTPVFADGTLAELNMKTVAGSVTIEPSQPVKTVTATVGTATVKSGETVAVPVTLSNVPGIATAELQVGFDATLLEVASITVGDIVLNPSVNFSSVVNGSTIKLLFLDDTLGSQLISKDGVLATINFKAKTVTSKVTTPVAVSGTPVFADGTLAELKYETVAGSVTIEPSQPVKTVTATVGTATGKVGETVAVPVTLSNVPGIATAEVQVGFDATLLEVASITAGDIVLNPSVNFSSVVNGSTIKILFLDDTLGSQLISKDGVFATINFKIKAVPSTGTTPVAISGTPVFADGTLAEVQYKTVAGSVTIAAADIKAVKATVGTATGKAGDTVAVPVTLSNVSGIATVELQLSFDATLLEVASITAGDIVLNPSVNFSSVVNGSTIKILFLDDTLGSQLISKDGVFATVNFKVKSTATNSAVTPVTVSGTPVFADGTLAELKSESAAGRLTILPTVIIVDSTVAPTAVTFDKANQADAAITMTLNGNTFSAIKNGTATLVKGTDYTVSENVVTISKAYLAKQTGTVTLEFVFDKGNSAKVVVAVKEIQIVNSTITPVVATFEKTAAKQADVVVTMSLNGNTFSAIKNGTTTLVKGTDYTISGSTVTISKAYLATLADGSATLEFVFNQGASAKLRLTIVPAVVDPVVTDFAVKIDKVSAAAGSTVKVPVSLINVSKVGNVCVAEYKISFDSSVLTYVGTTAGTSIKNPAVNFSSQLNGNTITLLFFDNTIGNELITADGQFATIEFKVNAAATSGTTAEVKVATISSFADASLTEITKVATVNGSVKVS